European Patent Application EP 4 455 142 A1, published October 30, 2024. Title: Novel inhibitor of QPCTL and/or QC. Applicant: Scenic Immunology B.V. The sequence listing filed with the application follows.

SEQUENCE LISTING (3 sequences)

SEQ ID NO: 1 - DNA, 427 bp, synthetic construct
  source 1..427: mol_type = other DNA; note = synthetic DNA fragment
cagggacagcagagatccagtttggttaattaaggtaccgagggcctatttcccatgattccttcatatttgcatatacgatacaaggctgttagagagataattagaattaatttgactgtaaacacaaagatattagtacaaaatacgtgacgtagaaagtaataatttcttgggtagtttgcagttttaaaattatgttttaaaatggactatcatatgcttaccgtaacttgaaagtatttcgatttcttggctttatatatcttgtggaaaggacgaaacaccggagacggattaattaaaccgtctcagtttaagagctagaaatagcaagtttaaataaggctagtccgttatcaacttgaaaaagtggcaccgagtcggtgcttttttgaattcgctagctaggtcttgaaaggagtgg

SEQ ID NO: 2 - RNA, 75 nt, synthetic construct
  source 1..75: mol_type = other RNA; note = guide RNA targeting QPCTL
tatcttgtggaaaggacgaaacaccgcggggaggcttccgatcaatgtttaagagctagaaatagcaagtttaaa

SEQ ID NO: 3 - RNA, 75 nt, synthetic construct
  source 1..75: mol_type = other RNA; note = guide RNA targeting CD47
tatcttgtggaaaggacgaaacaccgctactgaagtatacgtaaaggtttaagagctagaaatagcaagtttaaa